European Patent Application EP 4 378 534 A2, published June 5, 2024. Title: Cyclotides as immunosuppressive agents. Applicant: Medizinische Universität Wien. The sequence listing filed with the application follows.

SEQUENCE LISTING (18 sequences)

SEQ ID NO: 1 - protein, 29 aa, Oldenlandia affinis
GLPVCGETCVGGTCNTPGCTCSWPVCTRN

SEQ ID NO: 2 - protein, 29 aa, Oldenlandia affinis
GLPVCGETCFGGTCNTPGCSCTWPICTRD

SEQ ID NO: 3 - protein, 29 aa, synthetic construct
  source 1..29: note = Mutant form of Kalata B1
  SITE 1: note = D-glycine
  SITE 2: note = D-leucine
  SITE 3: note = D-proline
  SITE 4: note = D-valine
  SITE 5: note = D-cysteine
  SITE 6: note = D-glycine
  SITE 7: note = D-glutamic acid
  SITE 8: note = D-threonine
  SITE 9: note = D-cysteine
  SITE 10: note = D-phenylalanine
  SITE 11..12: note = D-glycine
  SITE 13: note = D-threonine
  SITE 14: note = D-cysteine
  SITE 15: note = D-asparagine
  SITE 16: note = D-threonine
  SITE 17: note = D-proline
  SITE 18: note = D-glycine
  SITE 19: note = D-cysteine
  SITE 20: note = D-serine
  SITE 21: note = D-cysteine
  SITE 22: note = D-threonine
  SITE 23: note = D-tryptophan
  SITE 24: note = D-proline
  SITE 25: note = D-isoleucine
  SITE 26: note = D-cysteine
  SITE 27: note = D-threonine
  SITE 28: note = D-arginine
  SITE 29: note = D-aspartic acid
GLPVCGETCFGGTCNTPGCSCTWPICTRD

SEQ ID NO: 4 - protein, 29 aa, synthetic construct
  source 1..29: note = Mutant form of Kalata B1
GLPVCGETCVGGTCNTPKCTCSWPVCTRN

SEQ ID NO: 5 - protein, 29 aa, synthetic construct
  source 1..29: note = Mutant form of Kalata B1
GLPVCGETCVGGTCNTPGCTCSWPVCTRK

SEQ ID NO: 6 - protein, 29 aa, synthetic construct
  source 1..29: note = Mutant form of Kalata B1
KLPVCGETCVGGTCNTPGCKCSWPVCTRN

SEQ ID NO: 7 - protein, 29 aa, synthetic construct
  source 1..29: note = Mutant form of Kalata B1
GLPVCGETCVGGTCNTPGCKCSWPVCTRN

SEQ ID NO: 8 - protein, 29 aa, synthetic construct
  source 1..29: note = Mutant form of Kalata B1
GLPVCGEKCVGGTCNTPGCTCSWPVCTRN

SEQ ID NO: 9 - protein, 29 aa, synthetic construct
  source 1..29: note = Mutant form of Kalata B1
GLPVCGETCAGGTCNTPGCTCSWPVCTRN

SEQ ID NO: 10 - protein, 29 aa, synthetic construct
  source 1..29: note = Mutant form of Kalata B1
GLPVCGETCKGGTCNTPGCTCSWPVCTRN

SEQ ID NO: 11 - DNA, 87 bp, Oldenlandia affinis
  source 1..87: mol_type = unassigned DNA
ggacttccagtatgcggtgagacttgtgttgggggaacttgcaacactccaggctgcacttgctcctggcctgtttgcacacgcaat

SEQ ID NO: 12 - DNA, 87 bp, Oldenlandia affinis
  source 1..87: mol_type = unassigned DNA
ggtcttccagtatgcggcgagacttgctttgggggaacttgcaacactccaggctgctcttgcacctggcctatctgcacacgcgat

SEQ ID NO: 13 - protein, 124 aa, Oldenlandia affinis
MAKFTVCLLLCLLLAAFVGAFGSELSDSHKTTLVNEIAEKMLQRKILDGVEATLVTDVAEKMFLRKMKAEAKTSETADQVFLKQLQLKGLPVCGETCVGGTCNTPGCTCSWPVCTRNGLPSLAA

SEQ ID NO: 14 - protein, 210 aa, Oldenlandia affinis
MAKFTNCLVLSLLLAAFVGAFGAEFSEADKATLVNDIAENIQKEILGEVKTSETVLTMFLKEMQLKGLPVCGETCFGGTCNTPGCSCTWPICTRDSLPMRAGGKTSETTLHMFLKEMQLKGLPVCGETCFGGTCNTPGCSCTWPICTRDSLPMSAGGKTSETTLHMFLKEMQLKGLPVCGETCFGGTCNTPGCSCTWPICTRDSLPLVAA

SEQ ID NO: 15 - DNA, 724 bp, Oldenlandia affinis
  source 1..724: mol_type = unassigned DNA
ggcaccagcactttcttaaaatttactgctttttcttatttcttgttctgtgcttgcttcttccatggctaagttcaccgtctgtctcctcctgtgcttgcttcttgcagcatttgttggggcgtttggatctgagctttctgactcccacaagaccaccttggtcaatgaaatcgctgagaagatgctacaaagaaagatattggatggagtggaagctactttggtcactgatgtcgccgagaagatgttcctaagaaagatgaaggctgaagcgaaaacttctgaaaccgccgatcaggtgttcctgaaacagttgcagctcaaaggacttccagtatgcggtgagacttgtgttgggggaacttgcaacactccaggctgcacttgctcctggcctgtttgcacacgcaatggccttcctagtttggccgcataatttgcttgatcaaactgcaaaaatgaatgagaaggccgacaccaataaagctatcaatgtagttggtccctgtacttaatttggttggctccaaaccatgtgtgctgctcttgtttttgttttttcttttttcttctctctttcgggcactcttcaggacatgaagtgatgatcagtactctttgctatcatgttttctgtgcacaccttctattgtaggtgttgttgtgatgttgatgcccaattggaataaactgttgtcgttgttaaaaaaaaaaaaaaaaa

SEQ ID NO: 16 - DNA, 993 bp, Oldenlandia affinis
  source 1..993: mol_type = unassigned DNA
ggcaccagatacaacccctttcttataatttattgcttttcttattccttgaaaaaggagaaataatattggatcttccatggctaagttcaccaactgtctcgtcctgagcttgcttctagcagcatttgttggggctttcggagctgagttttctgaagccgacaaggccaccttggtcaatgatatcgctgagaatatccaaaaagagatactgggcgaagtgaagacttctgaaaccgtccttacgatgttcctgaaagagatgcagctcaaaggtcttccagtatgcggcgagacttgctttgggggaacttgcaacactccaggctgctcttgcacctggcctatctgcacacgcgatagccttcctatgagggctggaggaaaaacatctgaaaccacccttcatatgttcctgaaagagatgcagctcaagggtcttccagtttgcggcgagacttgctttgggggaacttgcaacactccaggctgctcgtgcacctggcctatctgcacacgcgatagccttcctatgagtgctggaggaaaaacatctgaaaccacccttcatatgttcctgaaagagatgcagctcaagggtcttccagtttgcggcgagacttgctttgggggaacttgcaacactccaggctgctcgtgcacctggcctatatgcacacgtgatagccttcctcttgtggctgcataatttgcttcatcaaactgcaaaatgaataagaagggacactaaattagctatgaattttgttggcccttgtgtctggtaatttggttcccgccaaattaaccatatgtatgcattgctccttttttctttcttttttttccccctcatttgggcactcttcattacatgaagagatcatgacgctttgttactctgagcaccccctgttggtgttgttcacatgttgatgcccatgttggaataaactcttgtttttgttaccaaaaaaaaaaaaaaaaaaa

SEQ ID NO: 17 - protein, 29 aa, synthetic construct
  VARIANT 1: note = X is A or R or N or D or C or Q or E or G or H or I or L or K or M or F or P or S or T or W or Y or V
  VARIANT 8: note = X is A or C or D or E or F or G or H or I or L or M or N or P or Q or R or S or T or V or W or Y
  VARIANT 10: note = X is C or D or E or F or G or H or I or L or M or N or P or Q or R or S or T or V or W or Y
  VARIANT 18..29: note = X is A or R or N or D or C or Q or E or G or H or I or L or K or M or F or P or S or T or W or Y or V
  source 1..29: note = Mutant form of Kalata B1
XLPVCGEXCXGGTCNTPXCXCXWPXCTRX

SEQ ID NO: 18 - protein, 21 aa, unidentified
  source 1..21: note = encephalitogenic peptide MOG35-55
MEVGWYRSPFSRVVHLYRNGK